European Patent Specification EP 3 509 575 B1, published March 19, 2025. Title: COMPOSITIONS AND METHODS FOR TREATMENT OF INSULIN RESISTANCE. Applicant: Temple University - of the Commonwealth System of Higher Education Merali, Salim Barrero, Carlos A. Childers, Wayne E. Morton, George C. The sequence listing filed with the application follows.

SEQUENCE LISTING (2 sequences)

SEQ ID NO: 1 - protein, 18 aa, Homo sapiens
  MISC_FEATURE (1)..(18): fragment of GLUT4 (amino acids 247-264)
LTGWADVSGVLAELKDEK

SEQ ID NO: 2 - protein, 18 aa, Artificial Sequence
  Adduct synthetically prepared
  MOD_RES (18)..(18): GLUT4-K264-NHE-adduct: 4-NHE adduct linked to terminal lysine (corresponds to lysine 264 of GLUT4)
LTGWADVSGVLAELKDEK